European Patent Specification EP 3 751 006 B1, published April 24, 2024. Title: NUCLEIC ACID AMPLIFICATION METHOD. Applicant: AB Analitica s.r.l. The sequence listing filed with the application follows.

SEQUENCE LISTING (11 sequences)

SEQ ID NO: 1 - DNA, 197 bp, Artificial Sequence
  Pan Control
aaacctgtcttgtaaccttgataccaacctgcccagggcctcaccaccaacttcatccacgttcacctaaacaatccggaagcgaccaacgccttgattgacaaggatggatggctacattctggagacatagcttctcctcaggagtcaggtgcaccatggtgtctgtttgaggttgctagtgaacacagttgtgt

SEQ ID NO: 2 - DNA, 21 bp, Artificial Sequence
  primer
ctcgaatccaacggatttgac

SEQ ID NO: 3 - DNA, 19 bp, Artificial Sequence
  primer
ggcacgctattctgcagca

SEQ ID NO: 4 - DNA, 19 bp, Artificial Sequence
  probe
ccatggtcgtgccgcagca

SEQ ID NO: 5 - DNA, 24 bp, Artificial Sequence
  primer
cctgtcttgtaaccttgataccaa

SEQ ID NO: 6 - DNA, 20 bp, Artificial Sequence
  primer
atggtgcagctgactcctga

SEQ ID NO: 7 - DNA, 23 bp, Artificial Sequence
  probe
atccacgttcaccttgccccaca

SEQ ID NO: 8 - DNA, 27 bp, Artificial Sequence
  probe
acgccttgattgacaaggatggatggc

SEQ ID NO: 9 - DNA, 20 bp, Artificial Sequence
  primer
ccacactaggagagcagact

SEQ ID NO: 10 - DNA, 17 bp, Artificial Sequence
  primer
gccaagcggcctctgat

SEQ ID NO: 11 - DNA, 18 bp, Artificial Sequence
  probe
gcatgaaggtctttgccc